European Patent Specification EP 3 969 581 B1, published October 8, 2025. Title: CAPTURE AND ANALYSIS OF TARGET GENOMIC REGIONS. Applicant: RAPiD Genomics LLC. The sequence listing filed with the application follows.

SEQUENCE LISTING (9 sequences)

SEQ ID NO: 1 - DNA, 401 bp, Artificial Sequence
  synthetic
  misc_feature (75)..(75): n = Ala or Gly
  misc_feature (176)..(176): n = Gly or Ala
  misc_feature (250)..(250): n = Thr or Cys
  misc_feature (300)..(300): n = Cys or Gly
acccactgttgagagtcagtggcaagagaagtctcgtcttttacgtcccgtatcaaaatgagtgtacaatacatntctatgtgcgagtgagagcacgggtctgggcctggagagtggaccacctacaattggccatttcggtttgcggaagctgtcaagtcaacgcgagtcctagnatctcatagtcttcgcattaacccgtattaagtggactcgcctacagtttgtcttatgctagcaacccaggcanagtctgtacgcgcgatcgtccactggtagtggggtccttcctggagtgtngtatgggccatccggtctaccttactaacttaggctttaagcgcatttctatgtgcgtgaggtgtcgcattcatacttagtctggtcctaagtctgtcacc

SEQ ID NO: 2 - DNA, 20 bp, Artificial Sequence
  synthetic
tctatgtgcgagtgagagca

SEQ ID NO: 3 - DNA, 20 bp, Artificial Sequence
  synthetic
gcgcgatcgtccactggtag

SEQ ID NO: 4 - DNA, 184 bp, Artificial Sequence
  synthetic
  misc_feature (84)..(84): n = Gly or Ala
  misc_feature (158)..(158): n = Thr or Cys
gcacgggtctgggcctggagagtggaccacctacaattggccatttcggtttgcggaagctgtcaagtcaacgcgagtcctagnatctcatagtcttcgcattaacccgtattaagtggactcgcctacagtttgtcttatgctagcaacccaggcanagtctgtacgcgcgatcgtccactgg

SEQ ID NO: 5 - DNA, 30 bp, Artificial Sequence
  synthetic
gcacgggtctgggcctggagagtggaccac

SEQ ID NO: 6 - DNA, 30 bp, Artificial Sequence
  synthetic
gcatagtctgtacgcgcgatcgtccactgg

SEQ ID NO: 7 - DNA, 30 bp, Artificial Sequence
  synthetic
gtggtccactctccaggcccagacccgtgc

SEQ ID NO: 8 - DNA, 30 bp, Artificial Sequence
  synthetic
ccagtggacgatcgcgcgtacagactatgc

SEQ ID NO: 9 - DNA, 60 bp, Artificial Sequence
  synthetic
gtggtccactctccaggcccagacccgtgcccagtggacgatcgcgcgtacagactatgc